European Patent Application EP 4 302 593 A1, published January 10, 2024. Title: Solanaceae plant and solanaceae plant cells resistant to Begomovirus causing yellow leaf curling symptoms in tomato and method for producing such solanaceae plant. Applicant: Kikkoman Corporation National University Corporation Hokkaido University Atarashi, Hiroki Kwon, Joon Nakahara, Kenji. The sequence listing filed with the application follows.

SEQUENCE LISTING (42 sequences)

SEQ ID NO: 1 - DNA, 4586 bp, Solanum lycopersicum
  misc_feature (1)..(4586): cDNA sequence of DCL3 gene
  misc_feature (1089)..(1348): Exon 8
  misc_feature (1308)..(1327): Target sequence
atggcgacatcaacttgtgagctaatttggctcaaacagttgctgagagagctaaaatttggcgaaattaatcagatggaacttgtgtgtgataatcaagcggctctttatatcgcatcaaatctatttgatgctgcattagctgatttgaaactgtcactgccaagtcagtacaaagatacagatgatatatataagaagcttcggaagagattgtccaattgttatgcaaagatattgtgttgccttgaaaatctaggcatcatttgtgcttatgaggctgttaaaatctgcttggaaaatgtgcctaatgacaaagatgaaaatgagattctaaggacaagttctctacaacatagatacttcttggaggaggcattgtcaattgtccaggaatcaatgccacaagactgtgagagcctcttcgatgttggatatgacttgtcagcaactctgtcaatgggccatatatcttcaaaactgcaagtgcttcttgaaatttttcaactccttgggaaagccactcaagtacgctgtctcatttttgttgaaagaattataacagctaaggttattgaaagagttatgaagaaaatgacctggttttcacatttcacaatagcatatttgactggaacaaacacatcggtcgatgctctgacacgaaaagcgcaaaaagaaaccttgggatcttttctctctggaaaggtcaatttattatttgccactgatgtggttgaggagggaattgatgtgccacactgttcctctgtaatacgatttgatttacccaagacagttcgtagttatgtccaatctaggggacgtgctcgtcagactgagtctcagtatatactaatgcttgagagaggaaacaagaagcagagggagcagatgttcgatattatcaggagtgaatattctatgacagatacagctataaagagagatcctgatgattctgtggtgaaaccttgtcttgtgaaggaaactaaagcatattatgtggaggcaactggagcatcagtaactgcagattctagtgtcagtgtcttgactaaatattgtgaaatgctccctggagataaattcttctctccaaagccagtgtttcagtacattttgtctggagagttgtaccggtgtaagttgacattacctccaaatgcagctctccaaacgattgttggtccagaatgcaggagttctcaactatcaaggcagcttgtctgcttggatgcatgtaagaagctgcaccagattggtgctctcaatgaccatcttcttcctttcaatgaaaaacctccccgaggtggctctgatgtgcaggacagaaaattaggcgcaggaacaacaaagttgaaagaattacatgggacagcttgtattagtgcattatctgggtcatggggaaatgatcctaatggagaagtatatcaagtgtataaaatgaacttcctttgcaacatcaaggaagttaaatattccagttttatccttttgcttcaatcagaacttgattacgatgtgggaaatgtggaagtggagcttttcttagtttccaagtttgtcgaatcctctgtgtcgcattgtgggaaagtacatttggattcccaacaggtggcaaaagcaaaaatattccaagaactattctttaatgggctgtttggtaaattatttattaaatcatcgtgtggaaggaaatttctgcttgatacagaaaaatctttgtgggagccatcgaacatgtacttgcttctaccgctggatcctttagattcaagttgtgaaccctacagagttgattgggaagcaattgaatcttctgtttcagttgtagaatttttgaaaaaaaatgggtggttaagcaaggagaaatctgaagctaaacggaagaactccttagttgataggactgcatcatttgtggaagatattgatcaaaccgatttgattcactttgccaatatgtcaatctcaagaagcaagattatggacatggttgttgtggccattcatactggaagaatttattctgttctggaggctgttgccaattcttccgcagagagccccttcgaagttgattcagaagctactgtagccccgttctcatcttttgctgactacttccataaaaagtacgggattgttttagtgtatcctggacagcctttgttgctactgaagcaaagccataacgcatacaatcttctcgtggattttaaaaaggaaggtatttcatgtggaccgaaatcaaaagatagtacaatggtggttaaaaagccactgaataatgttcatatgccaccagaacttctggtctgttttgacattcggttagacatcttgaaatccttctacttgctaccatcattaatgcaccgcctggcgtccctgatgttggctagccagttgaggaaagatatatcaagccattcaggggacttacatatatcaagctcattgattctggaagctcttacaactctcagatgcaatgagagtttctccatggaacgtctggagttgcttggagattctgttctgaaatatgctgttagttgttacctcttccttaaatatcccaagaagcatgaagggcagctaactaatgaacgttcacaggctattagtaactcagccctccataaattgggaactaatcaacatttgcagggttatatacgggatggcgcatttgatccacgccgatggactgctcctgggcagctttccctgtggctttgtccttgtgaacacggggttgaaacttcacaagtgcctttggacaagaagtttctgactgaagatcccaaagaagtagttgggaagcactgtgatagaggacacagatggatgggttcaaaaactatatctgactgtgttgaagcgttaataggtgcatattacgttggtggtgggtttgttgctgccctcaaattgatgaaatggcttggttttaaagctgagctagaaccttcattagtagaagatgcgatcaatactgcatctctttattcttatacccctaaagctaaagatattgaagaccttgagttgaagcttgcttataaattttctattaagggactgcttttagaagctataacacacgctactgtgcaagagctggaggctgggtacagttatcagaggcttgaatttcttggcgactcagtactggacattctcgttacctggtacctttaccagaagcacaaagatattgatcctggggaactaacagatctgcgttctgcttctgtcaataatgataatttcgcttatgctgctgtgagaaggaatcttcatgtccaccttcaacatcattctggatgtcttgaaagtgaaatatcattatttgtgaagtcagtctctaattccgattcactccaaggaaacaaagccccaaaggtacttggagacttggtggagagtattgctggagcagtacttattgataccaagcttaacctggatgaagtttggaagatcttcaagccactgttgtctcccatcgtgactcctgataagcttgaactacctccattccgtgagctcatagaattatgtgactcacttggctacttctttaaagaacattgtgtgatgaagggggataccgtaaatgctgagcttaggttacagctgatagatgatctgctgatcgctgagggatctgggcaaactagaaaaaatgcaaaggcgcaagcagctctgaagttactgaagaacttagagaaaaaaggaatttcatttaagaagaaaaaagaagaggccagctttgttgatgtgccacaatctttagactttgatggtgacatctgcatccaagcaaatacttcttgtcctgatatggcttcacgcaaaaagcgaaagaaagtatatttgaataataagacggatgaagctcaatctgttcccagtgactgctccaccagttctagctattcaaataaggacacccaagtaattgggccaatcaacatgacaaggggtggacctcgcatatcactctttgaactatgcaagaaactgcagtggccaatgcctagttttgaatcaacagagcgtacatccaaatcacttattgaatgtggtgaaggctctgataaaaggaaggtttacaacacttttgcatctcgaatctctctgacaatacctgactatggtttgatagagcttaccggggatgaaagagctgataagaaaagctcacttgattcagcagcacttcacatgttatatgagctagaacgacaggggaaaatagccattggaaatcaatgaattatcattagtgtgaattctcacaatcttgctctaaggcgtagaattgttagcatatagccttttaggtctagcccttcgctaagggaatccagaaattgctgtgtatatttgcattgaaaagtagcaacaaacttagtagtagcgtatcaggcgggcatggtttctgtttccagccattattggaaatccaattgaaaatagggatgaactttttgaagtgtataacggggattgttcttatgtcccttatttaaaccttgatttaacttatctattgggacttccttctt

SEQ ID NO: 2 - DNA, 260 bp, Solanum lycopersicum
  misc_feature (1)..(260): Exon 8 of DCL3 gene
  misc_feature (220)..(239): Target sequence
attcttctctccaaagccagtgtttcagtacattttgtctggagagttgtaccggtgtaagttgacattacctccaaatgcagctctccaaacgattgttggtccagaatgcaggagttctcaactatcaaggcagcttgtctgcttggatgcatgtaagaagctgcaccagattggtgctctcaatgaccatcttcttcctttcaatgaaaaacctccccgaggtggctctgatgtgcaggacagaaaattaggcgcag

SEQ ID NO: 3 - DNA, 20 bp, Solanum lycopersicum
  misc_feature (1)..(20): Target sequence of exon 8 of DCL3 gene
ccgaggtggctctgatgtgc

SEQ ID NO: 4 - DNA, 1960 bp, Solanum lycopersicum
  misc_feature (1)..(1960): cDNA sequence of 4CL06 gene
  misc_feature (669)..(1136): Exon 2
  misc_feature (954)..(973): Target sequence
caggacacctaaaaaagtcttcaacactttttctttattgctcttagcgagcccaaaatttcaaactatagtactacattttttttttattcttcttctcgtcaagtctcaaaagctaaatcaaaatgacaaatgcaacgatggagaacgaaacaaaacaagacgatataatttttcgatcgaagctccctgatatttacatccctaatcatcttccgttacactcgtattgtttcgaaaatatttcggaattcaaatcgcgcccgtgtttaatcgacggggcgaataatcaaatttatacatacgctgatgttgagctcaattcgagaaaagttgctgctggtcttcataaacaatttgggatccaacaaaaggatactattatgatcttattgccaaattcaccagaatttgtgtatgtcttccttggtgcgtcgtacctcggcgcgatatcgacgatggctaatcctttgtttacgtctgctgaagttgtgaagcaagctaaggcttctaatgctaagatcattgtcactcaatcgtgtcatgtgaacaaggtgaaggattatgcattggagaatggtgtgaagatcgtgtgtatcgatccggcccctgacggttgtgttcacttttctgagttgattcaggccgatgagcatgatatccctgaggtgaaaatccaacccgatgatgtggtggcgttgccgtattcctccggaacaacgggtttacctaaaggtgtcatgttgacacacaagggactagtcacaagtgtggcacaacaagttgatggtgaaaatccaaacttgtacatccatagtgaggatgtattgctttgtgtgttgcctttgtttcatatatattccctcaattccgttttgctatgtggattaagagttggagcagcaattttgattatgcaaaaatttgacattgttccattcttggaattaatacaaaattacaaggtgaccatagggccatttgtgccacctattgttttggctattgctaagagtcctatggttgataattatgatttatcatcggtaagaaccgttatgtctggggctgcaccattaggaaaagaacttgaagacactgttcgagccaaatttcctaatgctaaacttggtcaaggttacggaatgacagaagccggaccagtgttggctatgtgcttggcatttgctaaagaacccttcgaaattaaatctggagcatgtgggactgttgttagaaatgctcagatgaaaattgtggatcctgatactggcaaatctctccctaggaaccaatctggagagatttgtataagaggcgatcaaattatgaaaggttacctaaatgatccagaggccactacgggaacaatagacaaagaaaggtggttacatacgggcgatattggttatattgacatcgatgatgagcttttcattgtggatcgtttaaaggaattgataaaatacaaaggatttcaagtggctcctgctgaacttgaagcccttctcctcaatcatcccaatatttcagatgctgctgttgtttcaatgaaagacgagcaagcaggagaagttcctgtggcttttgttgtcagatcaaatggctccacaattactgaagatgaagtcaaagaattcataacaaagcaggtgatattctataaaaggataaagagggtattttttgtggatgttgttcctaaatctccatcgggcaaaatccttagaaaggacttgagagctaaattagctgctggatatccaaattaaatactacttcatactttaatggcgatcgaataactataaccaatatttttttttttgttattgaaagttacatatttttgttctttgaattgtatttgtacgttaaaccacctgcctctatacggttaaaattaattaaccaatttggcaaaaggagaaaaatgtatgtatatttgactgtaagggac

SEQ ID NO: 5 - DNA, 468 bp, Solanum lycopersicum
  misc_feature (1)..(468): Exon 2 of 4CL06 gene
  misc_feature (286)..(305): Target sequence
gtgaaaatccaacccgatgatgtggtggcgttgccgtattcctccggaacaacgggtttacctaaaggtgtcatgttgacacacaagggactagtcacaagtgtggcacaacaagttgatggtgaaaatccaaacttgtacatccatagtgaggatgtattgctttgtgtgttgcctttgtttcatatatattccctcaattccgttttgctatgtggattaagagttggagcagcaattttgattatgcaaaaatttgacattgttccattcttggaattaatacaaaattacaaggtgaccatagggccatttgtgccacctattgttttggctattgctaagagtcctatggttgataattatgatttatcatcggtaagaaccgttatgtctggggctgcaccattaggaaaagaacttgaagacactgttcgagccaaatttcctaatgctaaacttggtcaa

SEQ ID NO: 6 - DNA, 20 bp, Solanum lycopersicum
  misc_feature (1)..(468): Target sequence in exon 2 of 4CL06 gene
caaaattacaaggtgaccat

SEQ ID NO: 7 - DNA, 21 bp, Artificial Sequence
  Primer 1 for DCL3 gene
ctcaactatcaaggcagcttg

SEQ ID NO: 8 - DNA, 24 bp, Artificial Sequence
  Primer 2 for DCL3 gene
gataaaagctcctccttgccgagt

SEQ ID NO: 9 - DNA, 22 bp, Artificial Sequence
  Primer 3 for 4CL06 gene
ggtttacctaaaggtgtcatgt

SEQ ID NO: 10 - DNA, 22 bp, Artificial Sequence
  Primer 4 for 4CL06 gene
cagtgtcttcaagttcttttcc

SEQ ID NO: 11 - DNA, 20 bp, Artificial Sequence
  Primer 5 for TYLCV
ccctctggaatgaaggaaca

SEQ ID NO: 12 - DNA, 20 bp, Artificial Sequence
  Primer 6 for TYLCV
ttgaaaaattggrctctcaa

SEQ ID NO: 13 - DNA, 258 bp, Solanum lycopersicum
  misc_feature (1)..(258): Exon 8 of DCL3 gene with mutation D1
attcttctctccaaagccagtgtttcagtacattttgtctggagagttgtaccggtgtaagttgacattacctccaaatgcagctctccaaacgattgttggtccagaatgcaggagttctcaactatcaaggcagcttgtctgcttggatgcatgtaagaagctgcaccagattggtgctctcaatgaccatcttcttcctttcaatgaaaacctccccgaggtggctctgatggcaggacagaaaattaggcgcag

SEQ ID NO: 14 - DNA, 257 bp, Solanum lycopersicum
  misc_feature (1)..(257): Exon 8 of DCL3 gene with mutation D2
attcttctctccaaagccagtgtttcagtacattttgtctggagagttgtaccggtgtaagttgacattacctccaaatgcagctctccaaacgattgttggtccagaatgcaggagttctcaactatcaaggcagcttgtctgcttggatgcatgtaagaagctgcaccagattggtgctctcaatgaccatcttcttcctttcaatgaaaaacctccccgaggtggctctgtgcaggacagaaaattaggcgcag

SEQ ID NO: 15 - DNA, 259 bp, Solanum lycopersicum
  misc_feature (1)..(259): Exon 8 of DCL3 gene with mutation D3
attcttctctccaaagccagtgtttcagtacattttgtctggagagttgtaccggtgtaagttgacattacctccaaatgcagctctccaaacgattgttggtccagaatgcaggagttctcaactatcaaggcagcttgtctgcttggatgcatgtaagaagctgcaccagattggtgctctcaatgaccatcttcttcctttcaatgaaaaacctccccgaggtggctctgatggcaggacagaaaattaggcgcag

SEQ ID NO: 16 - DNA, 259 bp, Solanum lycopersicum
  misc_feature (1)..(259): Exon 8 of DCL3 gene with mutation D4
attcttctctccaaagccagtgtttcagtacattttgtctggagagttgtaccggtgtaagttgacattacctccaaatgcagctctccaaacgattgttggtccagaatgcaggagttctcaactatcaaggcagcttgtctgcttggatgcatgtaagaagctgcaccagattggtgctctcaatgaccatcttcttcctttcaatgaaaaacctccccgaggtggctctgatggcaagacagaaaattaggcgcag

SEQ ID NO: 17 - DNA, 258 bp, Solanum lycopersicum
  misc_feature (1)..(258): Exon 8 of DCL3 gene with mutation D5
attcttctctccaaagccagtgtttcagtacattttgtctggagagttgtaccggtgtaagttgacattacctccaaatgcagctctccaaacgattgttggtccagaatgcaggagttctcaactatcaaggcagcttgtctgcttggatgcatgtaagaagctgcaccagattggtgctctcaatgaccatcttcttcctttcaatgaaaaacctccccgaggtggctctgatgcaggacagaaaattaggcgcag

SEQ ID NO: 18 - DNA, 254 bp, Solanum lycopersicum
  misc_feature (1)..(254): Exon 8 of DCL3 gene with mutation D6
attcttctctccaaagccagtgtttcagtacattttgtctggagagttgtaccggtgtaagttgacattacctccaaatgcagctctccaaacgattgttggtccagaatgcaggagttctcaactatcaaggcagcttgtctgcttggatgcatgtaagaagctgcaccagattggtgctctcaatgaccatcttcttcctttcaatgaaaaacctccccgaggtggcttgcaggacagaaaattaggcgcag

SEQ ID NO: 19 - DNA, 467 bp, Solanum lycopersicum
  misc_feature (1)..(467): Exon 2 of 4CL06 gene with mutation G1
gtgaaaatccaacccgatgatgtggtggcgttgccgtattcctccggaacaacgggtttacctaaaggtgtcatgttgacacacaagggactagtcacaagtgtggcacaacaagttgatggtgaaaatccaaacttgtacatccatagtgaggatgtattgctttgtgtgttgcctttgtttcatatatattccctcaattccgttttgctatgtggattaagagttggagcagcaattttgattatgcaaaaatttgacattgttccattcttggaattaatacaaaattacaaggtgacatagggccatttgtgccacctattgttttggctattgctaagagtcctatggttgataattatgatttatcatcggtaagaaccgttatgtctggggctgcaccattaggaaaagaacttgaagacactgttcgagccaaatttcctaatgctaaacttggtcaa

SEQ ID NO: 20 - DNA, 417 bp, Solanum lycopersicum
  misc_feature (1)..(417): Exon 2 of 4CL06 gene with mutation G2
gtgaaaatccaacccgatgatgtggtggcgttgccgtattcctccggaacaacgggtttacctaaaggtgtcatgttgacacacaagggactagtcacaagtgtggcacaacaagttgatggtgaaaatccaaacttgtacatccatagtgaggatgtattgctttgtgtgttgcctttgtttcatatatattccctcaattccgttttgctatgtggattaagagttggagcagcaattttgattatgcaaaaatttgacattgtgccacctattgttttggctattgctaagagtcctatggttgataattatgatttatcatcggtaagaaccgttatgtctggggctgcaccattaggaaaagaacttgaagacactgttcgagccaaatttcctaatgctaaacttggtcaa

SEQ ID NO: 21 - DNA, 4584 bp, Solanum lycopersicum
  misc_feature (1)..(4584): cDNA sequence of DCL3 gene with mutation D1 in exon 8
atggcgacatcaacttgtgagctaatttggctcaaacagttgctgagagagctaaaatttggcgaaattaatcagatggaacttgtgtgtgataatcaagcggctctttatatcgcatcaaatctatttgatgctgcattagctgatttgaaactgtcactgccaagtcagtacaaagatacagatgatatatataagaagcttcggaagagattgtccaattgttatgcaaagatattgtgttgccttgaaaatctaggcatcatttgtgcttatgaggctgttaaaatctgcttggaaaatgtgcctaatgacaaagatgaaaatgagattctaaggacaagttctctacaacatagatacttcttggaggaggcattgtcaattgtccaggaatcaatgccacaagactgtgagagcctcttcgatgttggatatgacttgtcagcaactctgtcaatgggccatatatcttcaaaactgcaagtgcttcttgaaatttttcaactccttgggaaagccactcaagtacgctgtctcatttttgttgaaagaattataacagctaaggttattgaaagagttatgaagaaaatgacctggttttcacatttcacaatagcatatttgactggaacaaacacatcggtcgatgctctgacacgaaaagcgcaaaaagaaaccttgggatcttttctctctggaaaggtcaatttattatttgccactgatgtggttgaggagggaattgatgtgccacactgttcctctgtaatacgatttgatttacccaagacagttcgtagttatgtccaatctaggggacgtgctcgtcagactgagtctcagtatatactaatgcttgagagaggaaacaagaagcagagggagcagatgttcgatattatcaggagtgaatattctatgacagatacagctataaagagagatcctgatgattctgtggtgaaaccttgtcttgtgaaggaaactaaagcatattatgtggaggcaactggagcatcagtaactgcagattctagtgtcagtgtcttgactaaatattgtgaaatgctccctggagataaattcttctctccaaagccagtgtttcagtacattttgtctggagagttgtaccggtgtaagttgacattacctccaaatgcagctctccaaacgattgttggtccagaatgcaggagttctcaactatcaaggcagcttgtctgcttggatgcatgtaagaagctgcaccagattggtgctctcaatgaccatcttcttcctttcaatgaaaacctccccgaggtggctctgatggcaggacagaaaattaggcgcaggaacaacaaagttgaaagaattacatgggacagcttgtattagtgcattatctgggtcatggggaaatgatcctaatggagaagtatatcaagtgtataaaatgaacttcctttgcaacatcaaggaagttaaatattccagttttatccttttgcttcaatcagaacttgattacgatgtgggaaatgtggaagtggagcttttcttagtttccaagtttgtcgaatcctctgtgtcgcattgtgggaaagtacatttggattcccaacaggtggcaaaagcaaaaatattccaagaactattctttaatgggctgtttggtaaattatttattaaatcatcgtgtggaaggaaatttctgcttgatacagaaaaatctttgtgggagccatcgaacatgtacttgcttctaccgctggatcctttagattcaagttgtgaaccctacagagttgattgggaagcaattgaatcttctgtttcagttgtagaatttttgaaaaaaaatgggtggttaagcaaggagaaatctgaagctaaacggaagaactccttagttgataggactgcatcatttgtggaagatattgatcaaaccgatttgattcactttgccaatatgtcaatctcaagaagcaagattatggacatggttgttgtggccattcatactggaagaatttattctgttctggaggctgttgccaattcttccgcagagagccccttcgaagttgattcagaagctactgtagccccgttctcatcttttgctgactacttccataaaaagtacgggattgttttagtgtatcctggacagcctttgttgctactgaagcaaagccataacgcatacaatcttctcgtggattttaaaaaggaaggtatttcatgtggaccgaaatcaaaagatagtacaatggtggttaaaaagccactgaataatgttcatatgccaccagaacttctggtctgttttgacattcggttagacatcttgaaatccttctacttgctaccatcattaatgcaccgcctggcgtccctgatgttggctagccagttgaggaaagatatatcaagccattcaggggacttacatatatcaagctcattgattctggaagctcttacaactctcagatgcaatgagagtttctccatggaacgtctggagttgcttggagattctgttctgaaatatgctgttagttgttacctcttccttaaatatcccaagaagcatgaagggcagctaactaatgaacgttcacaggctattagtaactcagccctccataaattgggaactaatcaacatttgcagggttatatacgggatggcgcatttgatccacgccgatggactgctcctgggcagctttccctgtggctttgtccttgtgaacacggggttgaaacttcacaagtgcctttggacaagaagtttctgactgaagatcccaaagaagtagttgggaagcactgtgatagaggacacagatggatgggttcaaaaactatatctgactgtgttgaagcgttaataggtgcatattacgttggtggtgggtttgttgctgccctcaaattgatgaaatggcttggttttaaagctgagctagaaccttcattagtagaagatgcgatcaatactgcatctctttattcttatacccctaaagctaaagatattgaagaccttgagttgaagcttgcttataaattttctattaagggactgcttttagaagctataacacacgctactgtgcaagagctggaggctgggtacagttatcagaggcttgaatttcttggcgactcagtactggacattctcgttacctggtacctttaccagaagcacaaagatattgatcctggggaactaacagatctgcgttctgcttctgtcaataatgataatttcgcttatgctgctgtgagaaggaatcttcatgtccaccttcaacatcattctggatgtcttgaaagtgaaatatcattatttgtgaagtcagtctctaattccgattcactccaaggaaacaaagccccaaaggtacttggagacttggtggagagtattgctggagcagtacttattgataccaagcttaacctggatgaagtttggaagatcttcaagccactgttgtctcccatcgtgactcctgataagcttgaactacctccattccgtgagctcatagaattatgtgactcacttggctacttctttaaagaacattgtgtgatgaagggggataccgtaaatgctgagcttaggttacagctgatagatgatctgctgatcgctgagggatctgggcaaactagaaaaaatgcaaaggcgcaagcagctctgaagttactgaagaacttagagaaaaaaggaatttcatttaagaagaaaaaagaagaggccagctttgttgatgtgccacaatctttagactttgatggtgacatctgcatccaagcaaatacttcttgtcctgatatggcttcacgcaaaaagcgaaagaaagtatatttgaataataagacggatgaagctcaatctgttcccagtgactgctccaccagttctagctattcaaataaggacacccaagtaattgggccaatcaacatgacaaggggtggacctcgcatatcactctttgaactatgcaagaaactgcagtggccaatgcctagttttgaatcaacagagcgtacatccaaatcacttattgaatgtggtgaaggctctgataaaaggaaggtttacaacacttttgcatctcgaatctctctgacaatacctgactatggtttgatagagcttaccggggatgaaagagctgataagaaaagctcacttgattcagcagcacttcacatgttatatgagctagaacgacaggggaaaatagccattggaaatcaatgaattatcattagtgtgaattctcacaatcttgctctaaggcgtagaattgttagcatatagccttttaggtctagcccttcgctaagggaatccagaaattgctgtgtatatttgcattgaaaagtagcaacaaacttagtagtagcgtatcaggcgggcatggtttctgtttccagccattattggaaatccaattgaaaatagggatgaactttttgaagtgtataacggggattgttcttatgtcccttatttaaaccttgatttaacttatctattgggacttccttctt

SEQ ID NO: 22 - DNA, 4583 bp, Solanum lycopersicum
  misc_feature (1)..(4580): cDNA sequence of DCL3 gene with mutation D2 in exon 8
atggcgacatcaacttgtgagctaatttggctcaaacagttgctgagagagctaaaatttggcgaaattaatcagatggaacttgtgtgtgataatcaagcggctctttatatcgcatcaaatctatttgatgctgcattagctgatttgaaactgtcactgccaagtcagtacaaagatacagatgatatatataagaagcttcggaagagattgtccaattgttatgcaaagatattgtgttgccttgaaaatctaggcatcatttgtgcttatgaggctgttaaaatctgcttggaaaatgtgcctaatgacaaagatgaaaatgagattctaaggacaagttctctacaacatagatacttcttggaggaggcattgtcaattgtccaggaatcaatgccacaagactgtgagagcctcttcgatgttggatatgacttgtcagcaactctgtcaatgggccatatatcttcaaaactgcaagtgcttcttgaaatttttcaactccttgggaaagccactcaagtacgctgtctcatttttgttgaaagaattataacagctaaggttattgaaagagttatgaagaaaatgacctggttttcacatttcacaatagcatatttgactggaacaaacacatcggtcgatgctctgacacgaaaagcgcaaaaagaaaccttgggatcttttctctctggaaaggtcaatttattatttgccactgatgtggttgaggagggaattgatgtgccacactgttcctctgtaatacgatttgatttacccaagacagttcgtagttatgtccaatctaggggacgtgctcgtcagactgagtctcagtatatactaatgcttgagagaggaaacaagaagcagagggagcagatgttcgatattatcaggagtgaatattctatgacagatacagctataaagagagatcctgatgattctgtggtgaaaccttgtcttgtgaaggaaactaaagcatattatgtggaggcaactggagcatcagtaactgcagattctagtgtcagtgtcttgactaaatattgtgaaatgctccctggagataaattcttctctccaaagccagtgtttcagtacattttgtctggagagttgtaccggtgtaagttgacattacctccaaatgcagctctccaaacgattgttggtccagaatgcaggagttctcaactatcaaggcagcttgtctgcttggatgcatgtaagaagctgcaccagattggtgctctcaatgaccatcttcttcctttcaatgaaaaacctccccgaggtggctctgagcaggacagaaaattaggcgcaggaacaacaaagttgaaagaattacatgggacagcttgtattagtgcattatctgggtcatggggaaatgatcctaatggagaagtatatcaagtgtataaaatgaacttcctttgcaacatcaaggaagttaaatattccagttttatccttttgcttcaatcagaacttgattacgatgtgggaaatgtggaagtggagcttttcttagtttccaagtttgtcgaatcctctgtgtcgcattgtgggaaagtacatttggattcccaacaggtggcaaaagcaaaaatattccaagaactattctttaatgggctgtttggtaaattatttattaaatcatcgtgtggaaggaaatttctgcttgatacagaaaaatctttgtgggagccatcgaacatgtacttgcttctaccgctggatcctttagattcaagttgtgaaccctacagagttgattgggaagcaattgaatcttctgtttcagttgtagaatttttgaaaaaaaatgggtggttaagcaaggagaaatctgaagctaaacggaagaactccttagttgataggactgcatcatttgtggaagatattgatcaaaccgatttgattcactttgccaatatgtcaatctcaagaagcaagattatggacatggttgttgtggccattcatactggaagaatttattctgttctggaggctgttgccaattcttccgcagagagccccttcgaagttgattcagaagctactgtagccccgttctcatcttttgctgactacttccataaaaagtacgggattgttttagtgtatcctggacagcctttgttgctactgaagcaaagccataacgcatacaatcttctcgtggattttaaaaaggaaggtatttcatgtggaccgaaatcaaaagatagtacaatggtggttaaaaagccactgaataatgttcatatgccaccagaacttctggtctgttttgacattcggttagacatcttgaaatccttctacttgctaccatcattaatgcaccgcctggcgtccctgatgttggctagccagttgaggaaagatatatcaagccattcaggggacttacatatatcaagctcattgattctggaagctcttacaactctcagatgcaatgagagtttctccatggaacgtctggagttgcttggagattctgttctgaaatatgctgttagttgttacctcttccttaaatatcccaagaagcatgaagggcagctaactaatgaacgttcacaggctattagtaactcagccctccataaattgggaactaatcaacatttgcagggttatatacgggatggcgcatttgatccacgccgatggactgctcctgggcagctttccctgtggctttgtccttgtgaacacggggttgaaacttcacaagtgcctttggacaagaagtttctgactgaagatcccaaagaagtagttgggaagcactgtgatagaggacacagatggatgggttcaaaaactatatctgactgtgttgaagcgttaataggtgcatattacgttggtggtgggtttgttgctgccctcaaattgatgaaatggcttggttttaaagctgagctagaaccttcattagtagaagatgcgatcaatactgcatctctttattcttatacccctaaagctaaagatattgaagaccttgagttgaagcttgcttataaattttctattaagggactgcttttagaagctataacacacgctactgtgcaagagctggaggctgggtacagttatcagaggcttgaatttcttggcgactcagtactggacattctcgttacctggtacctttaccagaagcacaaagatattgatcctggggaactaacagatctgcgttctgcttctgtcaataatgataatttcgcttatgctgctgtgagaaggaatcttcatgtccaccttcaacatcattctggatgtcttgaaagtgaaatatcattatttgtgaagtcagtctctaattccgattcactccaaggaaacaaagccccaaaggtacttggagacttggtggagagtattgctggagcagtacttattgataccaagcttaacctggatgaagtttggaagatcttcaagccactgttgtctcccatcgtgactcctgataagcttgaactacctccattccgtgagctcatagaattatgtgactcacttggctacttctttaaagaacattgtgtgatgaagggggataccgtaaatgctgagcttaggttacagctgatagatgatctgctgatcgctgagggatctgggcaaactagaaaaaatgcaaaggcgcaagcagctctgaagttactgaagaacttagagaaaaaaggaatttcatttaagaagaaaaaagaagaggccagctttgttgatgtgccacaatctttagactttgatggtgacatctgcatccaagcaaatacttcttgtcctgatatggcttcacgcaaaaagcgaaagaaagtatatttgaataataagacggatgaagctcaatctgttcccagtgactgctccaccagttctagctattcaaataaggacacccaagtaattgggccaatcaacatgacaaggggtggacctcgcatatcactctttgaactatgcaagaaactgcagtggccaatgcctagttttgaatcaacagagcgtacatccaaatcacttattgaatgtggtgaaggctctgataaaaggaaggtttacaacacttttgcatctcgaatctctctgacaatacctgactatggtttgatagagcttaccggggatgaaagagctgataagaaaagctcacttgattcagcagcacttcacatgttatatgagctagaacgacaggggaaaatagccattggaaatcaatgaattatcattagtgtgaattctcacaatcttgctctaaggcgtagaattgttagcatatagccttttaggtctagcccttcgctaagggaatccagaaattgctgtgtatatttgcattgaaaagtagcaacaaacttagtagtagcgtatcaggcgggcatggtttctgtttccagccattattggaaatccaattgaaaatagggatgaactttttgaagtgtataacggggattgttcttatgtcccttatttaaaccttgatttaacttatctattgggacttccttctt

SEQ ID NO: 23 - DNA, 4585 bp, Solanum lycopersicum
  misc_feature (1)..(4585): cDNA sequence of DCL3 gene with mutation D3 in exon 8
atggcgacatcaacttgtgagctaatttggctcaaacagttgctgagagagctaaaatttggcgaaattaatcagatggaacttgtgtgtgataatcaagcggctctttatatcgcatcaaatctatttgatgctgcattagctgatttgaaactgtcactgccaagtcagtacaaagatacagatgatatatataagaagcttcggaagagattgtccaattgttatgcaaagatattgtgttgccttgaaaatctaggcatcatttgtgcttatgaggctgttaaaatctgcttggaaaatgtgcctaatgacaaagatgaaaatgagattctaaggacaagttctctacaacatagatacttcttggaggaggcattgtcaattgtccaggaatcaatgccacaagactgtgagagcctcttcgatgttggatatgacttgtcagcaactctgtcaatgggccatatatcttcaaaactgcaagtgcttcttgaaatttttcaactccttgggaaagccactcaagtacgctgtctcatttttgttgaaagaattataacagctaaggttattgaaagagttatgaagaaaatgacctggttttcacatttcacaatagcatatttgactggaacaaacacatcggtcgatgctctgacacgaaaagcgcaaaaagaaaccttgggatcttttctctctggaaaggtcaatttattatttgccactgatgtggttgaggagggaattgatgtgccacactgttcctctgtaatacgatttgatttacccaagacagttcgtagttatgtccaatctaggggacgtgctcgtcagactgagtctcagtatatactaatgcttgagagaggaaacaagaagcagagggagcagatgttcgatattatcaggagtgaatattctatgacagatacagctataaagagagatcctgatgattctgtggtgaaaccttgtcttgtgaaggaaactaaagcatattatgtggaggcaactggagcatcagtaactgcagattctagtgtcagtgtcttgactaaatattgtgaaatgctccctggagataaattcttctctccaaagccagtgtttcagtacattttgtctggagagttgtaccggtgtaagttgacattacctccaaatgcagctctccaaacgattgttggtccagaatgcaggagttctcaactatcaaggcagcttgtctgcttggatgcatgtaagaagctgcaccagattggtgctctcaatgaccatcttcttcctttcaatgaaaaacctccccgaggtggctctgatggcaggacagaaaattaggcgcaggaacaacaaagttgaaagaattacatgggacagcttgtattagtgcattatctgggtcatggggaaatgatcctaatggagaagtatatcaagtgtataaaatgaacttcctttgcaacatcaaggaagttaaatattccagttttatccttttgcttcaatcagaacttgattacgatgtgggaaatgtggaagtggagcttttcttagtttccaagtttgtcgaatcctctgtgtcgcattgtgggaaagtacatttggattcccaacaggtggcaaaagcaaaaatattccaagaactattctttaatgggctgtttggtaaattatttattaaatcatcgtgtggaaggaaatttctgcttgatacagaaaaatctttgtgggagccatcgaacatgtacttgcttctaccgctggatcctttagattcaagttgtgaaccctacagagttgattgggaagcaattgaatcttctgtttcagttgtagaatttttgaaaaaaaatgggtggttaagcaaggagaaatctgaagctaaacggaagaactccttagttgataggactgcatcatttgtggaagatattgatcaaaccgatttgattcactttgccaatatgtcaatctcaagaagcaagattatggacatggttgttgtggccattcatactggaagaatttattctgttctggaggctgttgccaattcttccgcagagagccccttcgaagttgattcagaagctactgtagccccgttctcatcttttgctgactacttccataaaaagtacgggattgttttagtgtatcctggacagcctttgttgctactgaagcaaagccataacgcatacaatcttctcgtggattttaaaaaggaaggtatttcatgtggaccgaaatcaaaagatagtacaatggtggttaaaaagccactgaataatgttcatatgccaccagaacttctggtctgttttgacattcggttagacatcttgaaatccttctacttgctaccatcattaatgcaccgcctggcgtccctgatgttggctagccagttgaggaaagatatatcaagccattcaggggacttacatatatcaagctcattgattctggaagctcttacaactctcagatgcaatgagagtttctccatggaacgtctggagttgcttggagattctgttctgaaatatgctgttagttgttacctcttccttaaatatcccaagaagcatgaagggcagctaactaatgaacgttcacaggctattagtaactcagccctccataaattgggaactaatcaacatttgcagggttatatacgggatggcgcatttgatccacgccgatggactgctcctgggcagctttccctgtggctttgtccttgtgaacacggggttgaaacttcacaagtgcctttggacaagaagtttctgactgaagatcccaaagaagtagttgggaagcactgtgatagaggacacagatggatgggttcaaaaactatatctgactgtgttgaagcgttaataggtgcatattacgttggtggtgggtttgttgctgccctcaaattgatgaaatggcttggttttaaagctgagctagaaccttcattagtagaagatgcgatcaatactgcatctctttattcttatacccctaaagctaaagatattgaagaccttgagttgaagcttgcttataaattttctattaagggactgcttttagaagctataacacacgctactgtgcaagagctggaggctgggtacagttatcagaggcttgaatttcttggcgactcagtactggacattctcgttacctggtacctttaccagaagcacaaagatattgatcctggggaactaacagatctgcgttctgcttctgtcaataatgataatttcgcttatgctgctgtgagaaggaatcttcatgtccaccttcaacatcattctggatgtcttgaaagtgaaatatcattatttgtgaagtcagtctctaattccgattcactccaaggaaacaaagccccaaaggtacttggagacttggtggagagtattgctggagcagtacttattgataccaagcttaacctggatgaagtttggaagatcttcaagccactgttgtctcccatcgtgactcctgataagcttgaactacctccattccgtgagctcatagaattatgtgactcacttggctacttctttaaagaacattgtgtgatgaagggggataccgtaaatgctgagcttaggttacagctgatagatgatctgctgatcgctgagggatctgggcaaactagaaaaaatgcaaaggcgcaagcagctctgaagttactgaagaacttagagaaaaaaggaatttcatttaagaagaaaaaagaagaggccagctttgttgatgtgccacaatctttagactttgatggtgacatctgcatccaagcaaatacttcttgtcctgatatggcttcacgcaaaaagcgaaagaaagtatatttgaataataagacggatgaagctcaatctgttcccagtgactgctccaccagttctagctattcaaataaggacacccaagtaattgggccaatcaacatgacaaggggtggacctcgcatatcactctttgaactatgcaagaaactgcagtggccaatgcctagttttgaatcaacagagcgtacatccaaatcacttattgaatgtggtgaaggctctgataaaaggaaggtttacaacacttttgcatctcgaatctctctgacaatacctgactatggtttgatagagcttaccggggatgaaagagctgataagaaaagctcacttgattcagcagcacttcacatgttatatgagctagaacgacaggggaaaatagccattggaaatcaatgaattatcattagtgtgaattctcacaatcttgctctaaggcgtagaattgttagcatatagccttttaggtctagcccttcgctaagggaatccagaaattgctgtgtatatttgcattgaaaagtagcaacaaacttagtagtagcgtatcaggcgggcatggtttctgtttccagccattattggaaatccaattgaaaatagggatgaactttttgaagtgtataacggggattgttcttatgtcccttatttaaaccttgatttaacttatctattgggacttccttctt

SEQ ID NO: 24 - DNA, 4585 bp, Solanum lycopersicum
  misc_feature (1)..(4585): cDNA sequence of DCL3 gene with mutation D4 in exon 8
atggcgacatcaacttgtgagctaatttggctcaaacagttgctgagagagctaaaatttggcgaaattaatcagatggaacttgtgtgtgataatcaagcggctctttatatcgcatcaaatctatttgatgctgcattagctgatttgaaactgtcactgccaagtcagtacaaagatacagatgatatatataagaagcttcggaagagattgtccaattgttatgcaaagatattgtgttgccttgaaaatctaggcatcatttgtgcttatgaggctgttaaaatctgcttggaaaatgtgcctaatgacaaagatgaaaatgagattctaaggacaagttctctacaacatagatacttcttggaggaggcattgtcaattgtccaggaatcaatgccacaagactgtgagagcctcttcgatgttggatatgacttgtcagcaactctgtcaatgggccatatatcttcaaaactgcaagtgcttcttgaaatttttcaactccttgggaaagccactcaagtacgctgtctcatttttgttgaaagaattataacagctaaggttattgaaagagttatgaagaaaatgacctggttttcacatttcacaatagcatatttgactggaacaaacacatcggtcgatgctctgacacgaaaagcgcaaaaagaaaccttgggatcttttctctctggaaaggtcaatttattatttgccactgatgtggttgaggagggaattgatgtgccacactgttcctctgtaatacgatttgatttacccaagacagttcgtagttatgtccaatctaggggacgtgctcgtcagactgagtctcagtatatactaatgcttgagagaggaaacaagaagcagagggagcagatgttcgatattatcaggagtgaatattctatgacagatacagctataaagagagatcctgatgattctgtggtgaaaccttgtcttgtgaaggaaactaaagcatattatgtggaggcaactggagcatcagtaactgcagattctagtgtcagtgtcttgactaaatattgtgaaatgctccctggagataaattcttctctccaaagccagtgtttcagtacattttgtctggagagttgtaccggtgtaagttgacattacctccaaatgcagctctccaaacgattgttggtccagaatgcaggagttctcaactatcaaggcagcttgtctgcttggatgcatgtaagaagctgcaccagattggtgctctcaatgaccatcttcttcctttcaatgaaaaacctccccgaggtggctctgatggcaagacagaaaattaggcgcaggaacaacaaagttgaaagaattacatgggacagcttgtattagtgcattatctgggtcatggggaaatgatcctaatggagaagtatatcaagtgtataaaatgaacttcctttgcaacatcaaggaagttaaatattccagttttatccttttgcttcaatcagaacttgattacgatgtgggaaatgtggaagtggagcttttcttagtttccaagtttgtcgaatcctctgtgtcgcattgtgggaaagtacatttggattcccaacaggtggcaaaagcaaaaatattccaagaactattctttaatgggctgtttggtaaattatttattaaatcatcgtgtggaaggaaatttctgcttgatacagaaaaatctttgtgggagccatcgaacatgtacttgcttctaccgctggatcctttagattcaagttgtgaaccctacagagttgattgggaagcaattgaatcttctgtttcagttgtagaatttttgaaaaaaaatgggtggttaagcaaggagaaatctgaagctaaacggaagaactccttagttgataggactgcatcatttgtggaagatattgatcaaaccgatttgattcactttgccaatatgtcaatctcaagaagcaagattatggacatggttgttgtggccattcatactggaagaatttattctgttctggaggctgttgccaattcttccgcagagagccccttcgaagttgattcagaagctactgtagccccgttctcatcttttgctgactacttccataaaaagtacgggattgttttagtgtatcctggacagcctttgttgctactgaagcaaagccataacgcatacaatcttctcgtggattttaaaaaggaaggtatttcatgtggaccgaaatcaaaagatagtacaatggtggttaaaaagccactgaataatgttcatatgccaccagaacttctggtctgttttgacattcggttagacatcttgaaatccttctacttgctaccatcattaatgcaccgcctggcgtccctgatgttggctagccagttgaggaaagatatatcaagccattcaggggacttacatatatcaagctcattgattctggaagctcttacaactctcagatgcaatgagagtttctccatggaacgtctggagttgcttggagattctgttctgaaatatgctgttagttgttacctcttccttaaatatcccaagaagcatgaagggcagctaactaatgaacgttcacaggctattagtaactcagccctccataaattgggaactaatcaacatttgcagggttatatacgggatggcgcatttgatccacgccgatggactgctcctgggcagctttccctgtggctttgtccttgtgaacacggggttgaaacttcacaagtgcctttggacaagaagtttctgactgaagatcccaaagaagtagttgggaagcactgtgatagaggacacagatggatgggttcaaaaactatatctgactgtgttgaagcgttaataggtgcatattacgttggtggtgggtttgttgctgccctcaaattgatgaaatggcttggttttaaagctgagctagaaccttcattagtagaagatgcgatcaatactgcatctctttattcttatacccctaaagctaaagatattgaagaccttgagttgaagcttgcttataaattttctattaagggactgcttttagaagctataacacacgctactgtgcaagagctggaggctgggtacagttatcagaggcttgaatttcttggcgactcagtactggacattctcgttacctggtacctttaccagaagcacaaagatattgatcctggggaactaacagatctgcgttctgcttctgtcaataatgataatttcgcttatgctgctgtgagaaggaatcttcatgtccaccttcaacatcattctggatgtcttgaaagtgaaatatcattatttgtgaagtcagtctctaattccgattcactccaaggaaacaaagccccaaaggtacttggagacttggtggagagtattgctggagcagtacttattgataccaagcttaacctggatgaagtttggaagatcttcaagccactgttgtctcccatcgtgactcctgataagcttgaactacctccattccgtgagctcatagaattatgtgactcacttggctacttctttaaagaacattgtgtgatgaagggggataccgtaaatgctgagcttaggttacagctgatagatgatctgctgatcgctgagggatctgggcaaactagaaaaaatgcaaaggcgcaagcagctctgaagttactgaagaacttagagaaaaaaggaatttcatttaagaagaaaaaagaagaggccagctttgttgatgtgccacaatctttagactttgatggtgacatctgcatccaagcaaatacttcttgtcctgatatggcttcacgcaaaaagcgaaagaaagtatatttgaataataagacggatgaagctcaatctgttcccagtgactgctccaccagttctagctattcaaataaggacacccaagtaattgggccaatcaacatgacaaggggtggacctcgcatatcactctttgaactatgcaagaaactgcagtggccaatgcctagttttgaatcaacagagcgtacatccaaatcacttattgaatgtggtgaaggctctgataaaaggaaggtttacaacacttttgcatctcgaatctctctgacaatacctgactatggtttgatagagcttaccggggatgaaagagctgataagaaaagctcacttgattcagcagcacttcacatgttatatgagctagaacgacaggggaaaatagccattggaaatcaatgaattatcattagtgtgaattctcacaatcttgctctaaggcgtagaattgttagcatatagccttttaggtctagcccttcgctaagggaatccagaaattgctgtgtatatttgcattgaaaagtagcaacaaacttagtagtagcgtatcaggcgggcatggtttctgtttccagccattattggaaatccaattgaaaatagggatgaactttttgaagtgtataacggggattgttcttatgtcccttatttaaaccttgatttaacttatctattgggacttccttctt

SEQ ID NO: 25 - DNA, 4584 bp, Solanum lycopersicum
  misc_feature (1)..(4584): cDNA sequence of DCL3 gene with mutation D5 in exon 8
atggcgacatcaacttgtgagctaatttggctcaaacagttgctgagagagctaaaatttggcgaaattaatcagatggaacttgtgtgtgataatcaagcggctctttatatcgcatcaaatctatttgatgctgcattagctgatttgaaactgtcactgccaagtcagtacaaagatacagatgatatatataagaagcttcggaagagattgtccaattgttatgcaaagatattgtgttgccttgaaaatctaggcatcatttgtgcttatgaggctgttaaaatctgcttggaaaatgtgcctaatgacaaagatgaaaatgagattctaaggacaagttctctacaacatagatacttcttggaggaggcattgtcaattgtccaggaatcaatgccacaagactgtgagagcctcttcgatgttggatatgacttgtcagcaactctgtcaatgggccatatatcttcaaaactgcaagtgcttcttgaaatttttcaactccttgggaaagccactcaagtacgctgtctcatttttgttgaaagaattataacagctaaggttattgaaagagttatgaagaaaatgacctggttttcacatttcacaatagcatatttgactggaacaaacacatcggtcgatgctctgacacgaaaagcgcaaaaagaaaccttgggatcttttctctctggaaaggtcaatttattatttgccactgatgtggttgaggagggaattgatgtgccacactgttcctctgtaatacgatttgatttacccaagacagttcgtagttatgtccaatctaggggacgtgctcgtcagactgagtctcagtatatactaatgcttgagagaggaaacaagaagcagagggagcagatgttcgatattatcaggagtgaatattctatgacagatacagctataaagagagatcctgatgattctgtggtgaaaccttgtcttgtgaaggaaactaaagcatattatgtggaggcaactggagcatcagtaactgcagattctagtgtcagtgtcttgactaaatattgtgaaatgctccctggagataaattcttctctccaaagccagtgtttcagtacattttgtctggagagttgtaccggtgtaagttgacattacctccaaatgcagctctccaaacgattgttggtccagaatgcaggagttctcaactatcaaggcagcttgtctgcttggatgcatgtaagaagctgcaccagattggtgctctcaatgaccatcttcttcctttcaatgaaaaacctccccgaggtggctctgatgcaggacagaaaattaggcgcaggaacaacaaagttgaaagaattacatgggacagcttgtattagtgcattatctgggtcatggggaaatgatcctaatggagaagtatatcaagtgtataaaatgaacttcctttgcaacatcaaggaagttaaatattccagttttatccttttgcttcaatcagaacttgattacgatgtgggaaatgtggaagtggagcttttcttagtttccaagtttgtcgaatcctctgtgtcgcattgtgggaaagtacatttggattcccaacaggtggcaaaagcaaaaatattccaagaactattctttaatgggctgtttggtaaattatttattaaatcatcgtgtggaaggaaatttctgcttgatacagaaaaatctttgtgggagccatcgaacatgtacttgcttctaccgctggatcctttagattcaagttgtgaaccctacagagttgattgggaagcaattgaatcttctgtttcagttgtagaatttttgaaaaaaaatgggtggttaagcaaggagaaatctgaagctaaacggaagaactccttagttgataggactgcatcatttgtggaagatattgatcaaaccgatttgattcactttgccaatatgtcaatctcaagaagcaagattatggacatggttgttgtggccattcatactggaagaatttattctgttctggaggctgttgccaattcttccgcagagagccccttcgaagttgattcagaagctactgtagccccgttctcatcttttgctgactacttccataaaaagtacgggattgttttagtgtatcctggacagcctttgttgctactgaagcaaagccataacgcatacaatcttctcgtggattttaaaaaggaaggtatttcatgtggaccgaaatcaaaagatagtacaatggtggttaaaaagccactgaataatgttcatatgccaccagaacttctggtctgttttgacattcggttagacatcttgaaatccttctacttgctaccatcattaatgcaccgcctggcgtccctgatgttggctagccagttgaggaaagatatatcaagccattcaggggacttacatatatcaagctcattgattctggaagctcttacaactctcagatgcaatgagagtttctccatggaacgtctggagttgcttggagattctgttctgaaatatgctgttagttgttacctcttccttaaatatcccaagaagcatgaagggcagctaactaatgaacgttcacaggctattagtaactcagccctccataaattgggaactaatcaacatttgcagggttatatacgggatggcgcatttgatccacgccgatggactgctcctgggcagctttccctgtggctttgtccttgtgaacacggggttgaaacttcacaagtgcctttggacaagaagtttctgactgaagatcccaaagaagtagttgggaagcactgtgatagaggacacagatggatgggttcaaaaactatatctgactgtgttgaagcgttaataggtgcatattacgttggtggtgggtttgttgctgccctcaaattgatgaaatggcttggttttaaagctgagctagaaccttcattagtagaagatgcgatcaatactgcatctctttattcttatacccctaaagctaaagatattgaagaccttgagttgaagcttgcttataaattttctattaagggactgcttttagaagctataacacacgctactgtgcaagagctggaggctgggtacagttatcagaggcttgaatttcttggcgactcagtactggacattctcgttacctggtacctttaccagaagcacaaagatattgatcctggggaactaacagatctgcgttctgcttctgtcaataatgataatttcgcttatgctgctgtgagaaggaatcttcatgtccaccttcaacatcattctggatgtcttgaaagtgaaatatcattatttgtgaagtcagtctctaattccgattcactccaaggaaacaaagccccaaaggtacttggagacttggtggagagtattgctggagcagtacttattgataccaagcttaacctggatgaagtttggaagatcttcaagccactgttgtctcccatcgtgactcctgataagcttgaactacctccattccgtgagctcatagaattatgtgactcacttggctacttctttaaagaacattgtgtgatgaagggggataccgtaaatgctgagcttaggttacagctgatagatgatctgctgatcgctgagggatctgggcaaactagaaaaaatgcaaaggcgcaagcagctctgaagttactgaagaacttagagaaaaaaggaatttcatttaagaagaaaaaagaagaggccagctttgttgatgtgccacaatctttagactttgatggtgacatctgcatccaagcaaatacttcttgtcctgatatggcttcacgcaaaaagcgaaagaaagtatatttgaataataagacggatgaagctcaatctgttcccagtgactgctccaccagttctagctattcaaataaggacacccaagtaattgggccaatcaacatgacaaggggtggacctcgcatatcactctttgaactatgcaagaaactgcagtggccaatgcctagttttgaatcaacagagcgtacatccaaatcacttattgaatgtggtgaaggctctgataaaaggaaggtttacaacacttttgcatctcgaatctctctgacaatacctgactatggtttgatagagcttaccggggatgaaagagctgataagaaaagctcacttgattcagcagcacttcacatgttatatgagctagaacgacaggggaaaatagccattggaaatcaatgaattatcattagtgtgaattctcacaatcttgctctaaggcgtagaattgttagcatatagccttttaggtctagcccttcgctaagggaatccagaaattgctgtgtatatttgcattgaaaagtagcaacaaacttagtagtagcgtatcaggcgggcatggtttctgtttccagccattattggaaatccaattgaaaatagggatgaactttttgaagtgtataacggggattgttcttatgtcccttatttaaaccttgatttaacttatctattgggacttccttctt

SEQ ID NO: 26 - DNA, 4580 bp, Solanum lycopersicum
  misc_feature (1)..(4580): cDNA sequence of DCL3 gene with mutation D6 in exon 8
atggcgacatcaacttgtgagctaatttggctcaaacagttgctgagagagctaaaatttggcgaaattaatcagatggaacttgtgtgtgataatcaagcggctctttatatcgcatcaaatctatttgatgctgcattagctgatttgaaactgtcactgccaagtcagtacaaagatacagatgatatatataagaagcttcggaagagattgtccaattgttatgcaaagatattgtgttgccttgaaaatctaggcatcatttgtgcttatgaggctgttaaaatctgcttggaaaatgtgcctaatgacaaagatgaaaatgagattctaaggacaagttctctacaacatagatacttcttggaggaggcattgtcaattgtccaggaatcaatgccacaagactgtgagagcctcttcgatgttggatatgacttgtcagcaactctgtcaatgggccatatatcttcaaaactgcaagtgcttcttgaaatttttcaactccttgggaaagccactcaagtacgctgtctcatttttgttgaaagaattataacagctaaggttattgaaagagttatgaagaaaatgacctggttttcacatttcacaatagcatatttgactggaacaaacacatcggtcgatgctctgacacgaaaagcgcaaaaagaaaccttgggatcttttctctctggaaaggtcaatttattatttgccactgatgtggttgaggagggaattgatgtgccacactgttcctctgtaatacgatttgatttacccaagacagttcgtagttatgtccaatctaggggacgtgctcgtcagactgagtctcagtatatactaatgcttgagagaggaaacaagaagcagagggagcagatgttcgatattatcaggagtgaatattctatgacagatacagctataaagagagatcctgatgattctgtggtgaaaccttgtcttgtgaaggaaactaaagcatattatgtggaggcaactggagcatcagtaactgcagattctagtgtcagtgtcttgactaaatattgtgaaatgctccctggagataaattcttctctccaaagccagtgtttcagtacattttgtctggagagttgtaccggtgtaagttgacattacctccaaatgcagctctccaaacgattgttggtccagaatgcaggagttctcaactatcaaggcagcttgtctgcttggatgcatgtaagaagctgcaccagattggtgctctcaatgaccatcttcttcctttcaatgaaaaacctccccgaggtggcttgcaggacagaaaattaggcgcaggaacaacaaagttgaaagaattacatgggacagcttgtattagtgcattatctgggtcatggggaaatgatcctaatggagaagtatatcaagtgtataaaatgaacttcctttgcaacatcaaggaagttaaatattccagttttatccttttgcttcaatcagaacttgattacgatgtgggaaatgtggaagtggagcttttcttagtttccaagtttgtcgaatcctctgtgtcgcattgtgggaaagtacatttggattcccaacaggtggcaaaagcaaaaatattccaagaactattctttaatgggctgtttggtaaattatttattaaatcatcgtgtggaaggaaatttctgcttgatacagaaaaatctttgtgggagccatcgaacatgtacttgcttctaccgctggatcctttagattcaagttgtgaaccctacagagttgattgggaagcaattgaatcttctgtttcagttgtagaatttttgaaaaaaaatgggtggttaagcaaggagaaatctgaagctaaacggaagaactccttagttgataggactgcatcatttgtggaagatattgatcaaaccgatttgattcactttgccaatatgtcaatctcaagaagcaagattatggacatggttgttgtggccattcatactggaagaatttattctgttctggaggctgttgccaattcttccgcagagagccccttcgaagttgattcagaagctactgtagccccgttctcatcttttgctgactacttccataaaaagtacgggattgttttagtgtatcctggacagcctttgttgctactgaagcaaagccataacgcatacaatcttctcgtggattttaaaaaggaaggtatttcatgtggaccgaaatcaaaagatagtacaatggtggttaaaaagccactgaataatgttcatatgccaccagaacttctggtctgttttgacattcggttagacatcttgaaatccttctacttgctaccatcattaatgcaccgcctggcgtccctgatgttggctagccagttgaggaaagatatatcaagccattcaggggacttacatatatcaagctcattgattctggaagctcttacaactctcagatgcaatgagagtttctccatggaacgtctggagttgcttggagattctgttctgaaatatgctgttagttgttacctcttccttaaatatcccaagaagcatgaagggcagctaactaatgaacgttcacaggctattagtaactcagccctccataaattgggaactaatcaacatttgcagggttatatacgggatggcgcatttgatccacgccgatggactgctcctgggcagctttccctgtggctttgtccttgtgaacacggggttgaaacttcacaagtgcctttggacaagaagtttctgactgaagatcccaaagaagtagttgggaagcactgtgatagaggacacagatggatgggttcaaaaactatatctgactgtgttgaagcgttaataggtgcatattacgttggtggtgggtttgttgctgccctcaaattgatgaaatggcttggttttaaagctgagctagaaccttcattagtagaagatgcgatcaatactgcatctctttattcttatacccctaaagctaaagatattgaagaccttgagttgaagcttgcttataaattttctattaagggactgcttttagaagctataacacacgctactgtgcaagagctggaggctgggtacagttatcagaggcttgaatttcttggcgactcagtactggacattctcgttacctggtacctttaccagaagcacaaagatattgatcctggggaactaacagatctgcgttctgcttctgtcaataatgataatttcgcttatgctgctgtgagaaggaatcttcatgtccaccttcaacatcattctggatgtcttgaaagtgaaatatcattatttgtgaagtcagtctctaattccgattcactccaaggaaacaaagccccaaaggtacttggagacttggtggagagtattgctggagcagtacttattgataccaagcttaacctggatgaagtttggaagatcttcaagccactgttgtctcccatcgtgactcctgataagcttgaactacctccattccgtgagctcatagaattatgtgactcacttggctacttctttaaagaacattgtgtgatgaagggggataccgtaaatgctgagcttaggttacagctgatagatgatctgctgatcgctgagggatctgggcaaactagaaaaaatgcaaaggcgcaagcagctctgaagttactgaagaacttagagaaaaaaggaatttcatttaagaagaaaaaagaagaggccagctttgttgatgtgccacaatctttagactttgatggtgacatctgcatccaagcaaatacttcttgtcctgatatggcttcacgcaaaaagcgaaagaaagtatatttgaataataagacggatgaagctcaatctgttcccagtgactgctccaccagttctagctattcaaataaggacacccaagtaattgggccaatcaacatgacaaggggtggacctcgcatatcactctttgaactatgcaagaaactgcagtggccaatgcctagttttgaatcaacagagcgtacatccaaatcacttattgaatgtggtgaaggctctgataaaaggaaggtttacaacacttttgcatctcgaatctctctgacaatacctgactatggtttgatagagcttaccggggatgaaagagctgataagaaaagctcacttgattcagcagcacttcacatgttatatgagctagaacgacaggggaaaatagccattggaaatcaatgaattatcattagtgtgaattctcacaatcttgctctaaggcgtagaattgttagcatatagccttttaggtctagcccttcgctaagggaatccagaaattgctgtgtatatttgcattgaaaagtagcaacaaacttagtagtagcgtatcaggcgggcatggtttctgtttccagccattattggaaatccaattgaaaatagggatgaactttttgaagtgtataacggggattgttcttatgtcccttatttaaaccttgatttaacttatctattgggacttccttctt

SEQ ID NO: 27 - DNA, 1959 bp, Solanum lycopersicum
  misc_feature (1)..(1959): cDNA sequence of 4CL06 gene with mutation G1 in exon 2
caggacacctaaaaaagtcttcaacactttttctttattgctcttagcgagcccaaaatttcaaactatagtactacattttttttttattcttcttctcgtcaagtctcaaaagctaaatcaaaatgacaaatgcaacgatggagaacgaaacaaaacaagacgatataatttttcgatcgaagctccctgatatttacatccctaatcatcttccgttacactcgtattgtttcgaaaatatttcggaattcaaatcgcgcccgtgtttaatcgacggggcgaataatcaaatttatacatacgctgatgttgagctcaattcgagaaaagttgctgctggtcttcataaacaatttgggatccaacaaaaggatactattatgatcttattgccaaattcaccagaatttgtgtatgtcttccttggtgcgtcgtacctcggcgcgatatcgacgatggctaatcctttgtttacgtctgctgaagttgtgaagcaagctaaggcttctaatgctaagatcattgtcactcaatcgtgtcatgtgaacaaggtgaaggattatgcattggagaatggtgtgaagatcgtgtgtatcgatccggcccctgacggttgtgttcacttttctgagttgattcaggccgatgagcatgatatccctgaggtgaaaatccaacccgatgatgtggtggcgttgccgtattcctccggaacaacgggtttacctaaaggtgtcatgttgacacacaagggactagtcacaagtgtggcacaacaagttgatggtgaaaatccaaacttgtacatccatagtgaggatgtattgctttgtgtgttgcctttgtttcatatatattccctcaattccgttttgctatgtggattaagagttggagcagcaattttgattatgcaaaaatttgacattgttccattcttggaattaatacaaaattacaaggtgacatagggccatttgtgccacctattgttttggctattgctaagagtcctatggttgataattatgatttatcatcggtaagaaccgttatgtctggggctgcaccattaggaaaagaacttgaagacactgttcgagccaaatttcctaatgctaaacttggtcaaggttacggaatgacagaagccggaccagtgttggctatgtgcttggcatttgctaaagaacccttcgaaattaaatctggagcatgtgggactgttgttagaaatgctcagatgaaaattgtggatcctgatactggcaaatctctccctaggaaccaatctggagagatttgtataagaggcgatcaaattatgaaaggttacctaaatgatccagaggccactacgggaacaatagacaaagaaaggtggttacatacgggcgatattggttatattgacatcgatgatgagcttttcattgtggatcgtttaaaggaattgataaaatacaaaggatttcaagtggctcctgctgaacttgaagcccttctcctcaatcatcccaatatttcagatgctgctgttgtttcaatgaaagacgagcaagcaggagaagttcctgtggcttttgttgtcagatcaaatggctccacaattactgaagatgaagtcaaagaattcataacaaagcaggtgatattctataaaaggataaagagggtattttttgtggatgttgttcctaaatctccatcgggcaaaatccttagaaaggacttgagagctaaattagctgctggatatccaaattaaatactacttcatactttaatggcgatcgaataactataaccaatatttttttttttgttattgaaagttacatatttttgttctttgaattgtatttgtacgttaaaccacctgcctctatacggttaaaattaattaaccaatttggcaaaaggagaaaaatgtatgtatatttgactgtaagggac

SEQ ID NO: 28 - DNA, 1909 bp, Solanum lycopersicum
  misc_feature (1)..(1909): cDNA sequence of 4CL06 gene with mutation G2 in Exon 2
caggacacctaaaaaagtcttcaacactttttctttattgctcttagcgagcccaaaatttcaaactatagtactacattttttttttattcttcttctcgtcaagtctcaaaagctaaatcaaaatgacaaatgcaacgatggagaacgaaacaaaacaagacgatataatttttcgatcgaagctccctgatatttacatccctaatcatcttccgttacactcgtattgtttcgaaaatatttcggaattcaaatcgcgcccgtgtttaatcgacggggcgaataatcaaatttatacatacgctgatgttgagctcaattcgagaaaagttgctgctggtcttcataaacaatttgggatccaacaaaaggatactattatgatcttattgccaaattcaccagaatttgtgtatgtcttccttggtgcgtcgtacctcggcgcgatatcgacgatggctaatcctttgtttacgtctgctgaagttgtgaagcaagctaaggcttctaatgctaagatcattgtcactcaatcgtgtcatgtgaacaaggtgaaggattatgcattggagaatggtgtgaagatcgtgtgtatcgatccggcccctgacggttgtgttcacttttctgagttgattcaggccgatgagcatgatatccctgaggtgaaaatccaacccgatgatgtggtggcgttgccgtattcctccggaacaacgggtttacctaaaggtgtcatgttgacacacaagggactagtcacaagtgtggcacaacaagttgatggtgaaaatccaaacttgtacatccatagtgaggatgtattgctttgtgtgttgcctttgtttcatatatattccctcaattccgttttgctatgtggattaagagttggagcagcaattttgattatgcaaaaatttgacattgtgccacctattgttttggctattgctaagagtcctatggttgataattatgatttatcatcggtaagaaccgttatgtctggggctgcaccattaggaaaagaacttgaagacactgttcgagccaaatttcctaatgctaaacttggtcaaggttacggaatgacagaagccggaccagtgttggctatgtgcttggcatttgctaaagaacccttcgaaattaaatctggagcatgtgggactgttgttagaaatgctcagatgaaaattgtggatcctgatactggcaaatctctccctaggaaccaatctggagagatttgtataagaggcgatcaaattatgaaaggttacctaaatgatccagaggccactacgggaacaatagacaaagaaaggtggttacatacgggcgatattggttatattgacatcgatgatgagcttttcattgtggatcgtttaaaggaattgataaaatacaaaggatttcaagtggctcctgctgaacttgaagcccttctcctcaatcatcccaatatttcagatgctgctgttgtttcaatgaaagacgagcaagcaggagaagttcctgtggcttttgttgtcagatcaaatggctccacaattactgaagatgaagtcaaagaattcataacaaagcaggtgatattctataaaaggataaagagggtattttttgtggatgttgttcctaaatctccatcgggcaaaatccttagaaaggacttgagagctaaattagctgctggatatccaaattaaatactacttcatactttaatggcgatcgaataactataaccaatatttttttttttgttattgaaagttacatatttttgttctttgaattgtatttgtacgttaaaccacctgcctctatacggttaaaattaattaaccaatttggcaaaaggagaaaaatgtatgtatatttgactgtaagggac

SEQ ID NO: 29 - DNA, 1779 bp, Solanum lycopersicum
  misc_feature (1)..(1779): cDNA sequence of RLK2 gene
  misc_feature (1)..(830): Exon 1
  misc_feature (202)..(342): Deletion in Mutation 1
  misc_feature (269)..(280): Deletion in Mutation 2
  misc_feature (280)..(285): Deletion in Mutation 3
  misc_feature (277)..(296): Target sequence
gataaagacacatgaacttttcttcttctccaccatttctgctctgctctgctcactccaccattgaagaaacatgcgttttcttctcctcttcttccttactctaatactgcattttcatctcctccacttcaccaccgcaaaaccaccttacgtgccggaataccgcgcattgctctccctgaaaactgccattacagatgacccacaatctgctcttctttcatggaatatctccacaagtcattgtacatggagaggtgtcacgtgtgaccggtatcgtcacgtgacttctctcgacatatctggttttaatctcaccggtactcttacgccggaagttggtcatctccgttttttgctcaatctttctgtagctgttaaccagttctctggacccattcctgttgaactctcgtttataccaaatctgcgttaccttaacctctctaacaatattttcaacttgagtttccctccccagcttacccatctccggtacttgaatgttctcgacatttataataacaatatgaccggtgaacttcctgttggattttataatttgaccaatcttcgacatcttcatttgggtggcaatttttttagtggtagtattccaccggagtatggtagattcccattcctagaatatctggcagtttcgggaaatgcgctcgtcggtaggataccaccggagatcggaaatattaccacacttcgtgagctttacatcggatactacaacacgttttccggtgggttaccggcggaaatagggtacttgtcggagctcattcggttagatgctgcaaactgtggactttcaggaggtcacttgcattgggataccaggtataagatagcattggaggctgcaaagggactttgttatctccatcacgattgctcgcctctgatcctccatcgtgatgtaaaatcaaacaatatccttctggattccagcttcgaagcgcacgttgctgattttgggcttgccaagttcttgcaagactccggaacatcagaatgcatgtctgctattgctggttcttatggctacattgcaccagaatatgcatacacactcaaggtagatgagaagagtgatgtatacagctttggtgtggttctgttagaattggtgagcgggaaaaaaccggttggagaatttggtgatggcgttgacatagtccaatgggtaaggaggatgaccgatgggaaaaaggaaggagttctaaagatccttgatgcaagactctcaacagttccccttcatgaggtgatgcatgtgttctatgtcgcaatgctgtgtgtcgaagagcaagctgttgaacgccccaaaatgcgcgaggttgtgcaaatgttaactgagcttcccaagccatctggtccaaaatcaggagattcaacaatcaccgagtcgcccccttcatcaggtcctgcatcagagtctcctacttcgactcccagagacacaaaagaccagtaccatcatcagccaccacctcaatctcctccacctgaccttctcagcatatgacctgaaatgttcacttgtaatagagggtgtagttctcttctttaagttttattagtatcagttttattggggggttggtttattgtttaggctattagcttttcttaggaagtgtctcattgtacagtaagattggcagtaactttatccttcaaatttttccgtttgctttttagctttttgatattgaaagaatcccagtggtcaagctcaccactagccacttttcatcatta

SEQ ID NO: 30 - DNA, 830 bp, Solanum lycopersicum
  misc_feature (1)..(830): Exon 1 of RLK2 gene
  misc_feature (202)..(342): Deletion in Mutation 1
  misc_feature (269)..(280): Deletion in Mutation 2
  misc_feature (280)..(285): Deletion in Mutation 3
  misc_feature (277)..(296): Target sequence
gataaagacacatgaacttttcttcttctccaccatttctgctctgctctgctcactccaccattgaagaaacatgcgttttcttctcctcttcttccttactctaatactgcattttcatctcctccacttcaccaccgcaaaaccaccttacgtgccggaataccgcgcattgctctccctgaaaactgccattacagatgacccacaatctgctcttctttcatggaatatctccacaagtcattgtacatggagaggtgtcacgtgtgaccggtatcgtcacgtgacttctctcgacatatctggttttaatctcaccggtactcttacgccggaagttggtcatctccgttttttgctcaatctttctgtagctgttaaccagttctctggacccattcctgttgaactctcgtttataccaaatctgcgttaccttaacctctctaacaatattttcaacttgagtttccctccccagcttacccatctccggtacttgaatgttctcgacatttataataacaatatgaccggtgaacttcctgttggattttataatttgaccaatcttcgacatcttcatttgggtggcaatttttttagtggtagtattccaccggagtatggtagattcccattcctagaatatctggcagtttcgggaaatgcgctcgtcggtaggataccaccggagatcggaaatattaccacacttcgtgagctttacatcggatactacaacacgttttccggtgggttaccggcggaaatagggtacttgtcggagctcattcggttagatgctgcaaactgtggactttcag

SEQ ID NO: 31 - DNA, 20 bp, Solanum lycopersicum
  misc_feature (1)..(20): Target sequence in exon 1 of RLK2 gene
gtatcgtcacgtgacttctc

SEQ ID NO: 32 - DNA, 20 bp, Artificial Sequence
  Primer 1 for RLK2
ctccacttcaccaccgcaaa

SEQ ID NO: 33 - DNA, 20 bp, Artificial Sequence
  Primer 2 for RLK2
taccggagatgggtaagctg

SEQ ID NO: 34 - DNA, 689 bp, Solanum lycopersicum
  misc_feature (1)..(689): Exon 1 of RLK2 gene with mutation 1
gataaagacacatgaacttttcttcttctccaccatttctgctctgctctgctcactccaccattgaagaaacatgcgttttcttctcctcttcttccttactctaatactgcattttcatctcctccacttcaccaccgcaaaaccaccttacgtgccggaataccgcgcattgctctccctgaaaactgccattacagatggtcatctccgttttttgctcaatctttctgtagctgttaaccagttctctggacccattcctgttgaactctcgtttataccaaatctgcgttaccttaacctctctaacaatattttcaacttgagtttccctccccagcttacccatctccggtacttgaatgttctcgacatttataataacaatatgaccggtgaacttcctgttggattttataatttgaccaatcttcgacatcttcatttgggtggcaatttttttagtggtagtattccaccggagtatggtagattcccattcctagaatatctggcagtttcgggaaatgcgctcgtcggtaggataccaccggagatcggaaatattaccacacttcgtgagctttacatcggatactacaacacgttttccggtgggttaccggcggaaatagggtacttgtcggagctcattcggttagatgctgcaaactgtggactttcag

SEQ ID NO: 35 - DNA, 818 bp, Solanum lycopersicum
  misc_feature (1)..(818): Exon 1 of RLK2 gene with mutation 2
gataaagacacatgaacttttcttcttctccaccatttctgctctgctctgctcactccaccattgaagaaacatgcgttttcttctcctcttcttccttactctaatactgcattttcatctcctccacttcaccaccgcaaaaccaccttacgtgccggaataccgcgcattgctctccctgaaaactgccattacagatgacccacaatctgctcttctttcatggaatatctccacaagtcattgtacatggagaggtgtcacgtgtcacgtgacttctctcgacatatctggttttaatctcaccggtactcttacgccggaagttggtcatctccgttttttgctcaatctttctgtagctgttaaccagttctctggacccattcctgttgaactctcgtttataccaaatctgcgttaccttaacctctctaacaatattttcaacttgagtttccctccccagcttacccatctccggtacttgaatgttctcgacatttataataacaatatgaccggtgaacttcctgttggattttataatttgaccaatcttcgacatcttcatttgggtggcaatttttttagtggtagtattccaccggagtatggtagattcccattcctagaatatctggcagtttcgggaaatgcgctcgtcggtaggataccaccggagatcggaaatattaccacacttcgtgagctttacatcggatactacaacacgttttccggtgggttaccggcggaaatagggtacttgtcggagctcattcggttagatgctgcaaactgtggactttcag

SEQ ID NO: 36 - DNA, 141 bp, Artificial Sequence
  141 nucleotide deletion in Mutation 1
tgacccacaatctgctcttctttcatggaatatctccacaagtcattgtacatggagaggtgtcacgtgtgaccggtatcgtcacgtgacttctctcgacatatctggttttaatctcaccggtactcttacgccggaagt

SEQ ID NO: 37 - DNA, 12 bp, Artificial Sequence
  12 nucleotide deletion in Mutation 2
tgtgaccggtat

SEQ ID NO: 38 - DNA, 1638 bp, Solanum lycopersicum
  misc_feature (1)..(1638): cDNA sequence of mutated RLK2 gene of P15 line
  misc_feature (1)..(689): Exon 1 with mutation 1
gataaagacacatgaacttttcttcttctccaccatttctgctctgctctgctcactccaccattgaagaaacatgcgttttcttctcctcttcttccttactctaatactgcattttcatctcctccacttcaccaccgcaaaaccaccttacgtgccggaataccgcgcattgctctccctgaaaactgccattacagatggtcatctccgttttttgctcaatctttctgtagctgttaaccagttctctggacccattcctgttgaactctcgtttataccaaatctgcgttaccttaacctctctaacaatattttcaacttgagtttccctccccagcttacccatctccggtacttgaatgttctcgacatttataataacaatatgaccggtgaacttcctgttggattttataatttgaccaatcttcgacatcttcatttgggtggcaatttttttagtggtagtattccaccggagtatggtagattcccattcctagaatatctggcagtttcgggaaatgcgctcgtcggtaggataccaccggagatcggaaatattaccacacttcgtgagctttacatcggatactacaacacgttttccggtgggttaccggcggaaatagggtacttgtcggagctcattcggttagatgctgcaaactgtggactttcaggaggtcacttgcattgggataccaggtataagatagcattggaggctgcaaagggactttgttatctccatcacgattgctcgcctctgatcctccatcgtgatgtaaaatcaaacaatatccttctggattccagcttcgaagcgcacgttgctgattttgggcttgccaagttcttgcaagactccggaacatcagaatgcatgtctgctattgctggttcttatggctacattgcaccagaatatgcatacacactcaaggtagatgagaagagtgatgtatacagctttggtgtggttctgttagaattggtgagcgggaaaaaaccggttggagaatttggtgatggcgttgacatagtccaatgggtaaggaggatgaccgatgggaaaaaggaaggagttctaaagatccttgatgcaagactctcaacagttccccttcatgaggtgatgcatgtgttctatgtcgcaatgctgtgtgtcgaagagcaagctgttgaacgccccaaaatgcgcgaggttgtgcaaatgttaactgagcttcccaagccatctggtccaaaatcaggagattcaacaatcaccgagtcgcccccttcatcaggtcctgcatcagagtctcctacttcgactcccagagacacaaaagaccagtaccatcatcagccaccacctcaatctcctccacctgaccttctcagcatatgacctgaaatgttcacttgtaatagagggtgtagttctcttctttaagttttattagtatcagttttattggggggttggtttattgtttaggctattagcttttcttaggaagtgtctcattgtacagtaagattggcagtaactttatccttcaaatttttccgtttgctttttagctttttgatattgaaagaatcccagtggtcaagctcaccactagccacttttcatcatta

SEQ ID NO: 39 - DNA, 1767 bp, Solanum lycopersicum
  misc_feature (1)..(1767): cDNA sequence of mutated RLK2 gene of P24 line
  misc_feature (1)..(818): Exon 1 with mutation 2
gataaagacacatgaacttttcttcttctccaccatttctgctctgctctgctcactccaccattgaagaaacatgcgttttcttctcctcttcttccttactctaatactgcattttcatctcctccacttcaccaccgcaaaaccaccttacgtgccggaataccgcgcattgctctccctgaaaactgccattacagatgacccacaatctgctcttctttcatggaatatctccacaagtcattgtacatggagaggtgtcacgtgtcacgtgacttctctcgacatatctggttttaatctcaccggtactcttacgccggaagttggtcatctccgttttttgctcaatctttctgtagctgttaaccagttctctggacccattcctgttgaactctcgtttataccaaatctgcgttaccttaacctctctaacaatattttcaacttgagtttccctccccagcttacccatctccggtacttgaatgttctcgacatttataataacaatatgaccggtgaacttcctgttggattttataatttgaccaatcttcgacatcttcatttgggtggcaatttttttagtggtagtattccaccggagtatggtagattcccattcctagaatatctggcagtttcgggaaatgcgctcgtcggtaggataccaccggagatcggaaatattaccacacttcgtgagctttacatcggatactacaacacgttttccggtgggttaccggcggaaatagggtacttgtcggagctcattcggttagatgctgcaaactgtggactttcaggaggtcacttgcattgggataccaggtataagatagcattggaggctgcaaagggactttgttatctccatcacgattgctcgcctctgatcctccatcgtgatgtaaaatcaaacaatatccttctggattccagcttcgaagcgcacgttgctgattttgggcttgccaagttcttgcaagactccggaacatcagaatgcatgtctgctattgctggttcttatggctacattgcaccagaatatgcatacacactcaaggtagatgagaagagtgatgtatacagctttggtgtggttctgttagaattggtgagcgggaaaaaaccggttggagaatttggtgatggcgttgacatagtccaatgggtaaggaggatgaccgatgggaaaaaggaaggagttctaaagatccttgatgcaagactctcaacagttccccttcatgaggtgatgcatgtgttctatgtcgcaatgctgtgtgtcgaagagcaagctgttgaacgccccaaaatgcgcgaggttgtgcaaatgttaactgagcttcccaagccatctggtccaaaatcaggagattcaacaatcaccgagtcgcccccttcatcaggtcctgcatcagagtctcctacttcgactcccagagacacaaaagaccagtaccatcatcagccaccacctcaatctcctccacctgaccttctcagcatatgacctgaaatgttcacttgtaatagagggtgtagttctcttctttaagttttattagtatcagttttattggggggttggtttattgtttaggctattagcttttcttaggaagtgtctcattgtacagtaagattggcagtaactttatccttcaaatttttccgtttgctttttagctttttgatattgaaagaatcccagtggtcaagctcaccactagccacttttcatcatta

SEQ ID NO: 40 - DNA, 824 bp, Solanum lycopersicum
  misc_feature (1)..(824): Exon 1 of RLK2 gene with mutation 3
gataaagacacatgaacttttcttcttctccaccatttctgctctgctctgctcactccaccattgaagaaacatgcgttttcttctcctcttcttccttactctaatactgcattttcatctcctccacttcaccaccgcaaaaccaccttacgtgccggaataccgcgcattgctctccctgaaaactgccattacagatgacccacaatctgctcttctttcatggaatatctccacaagtcattgtacatggagaggtgtcacgtgtgaccggtacgtgacttctctcgacatatctggttttaatctcaccggtactcttacgccggaagttggtcatctccgttttttgctcaatctttctgtagctgttaaccagttctctggacccattcctgttgaactctcgtttataccaaatctgcgttaccttaacctctctaacaatattttcaacttgagtttccctccccagcttacccatctccggtacttgaatgttctcgacatttataataacaatatgaccggtgaacttcctgttggattttataatttgaccaatcttcgacatcttcatttgggtggcaatttttttagtggtagtattccaccggagtatggtagattcccattcctagaatatctggcagtttcgggaaatgcgctcgtcggtaggataccaccggagatcggaaatattaccacacttcgtgagctttacatcggatactacaacacgttttccggtgggttaccggcggaaatagggtacttgtcggagctcattcggttagatgctgcaaactgtggactttcag

SEQ ID NO: 41 - DNA, 6 bp, Artificial Sequence
  6 nucleotide deletion in Mutation 3
tcgtca

SEQ ID NO: 42 - DNA, 1773 bp, Solanum lycopersicum
  misc_feature (1)..(1773): cDNA sequence of mutated RLK2 gene of P19 line
  misc_feature (1)..(824): Exon 1 with mutation 3
gataaagacacatgaacttttcttcttctccaccatttctgctctgctctgctcactccaccattgaagaaacatgcgttttcttctcctcttcttccttactctaatactgcattttcatctcctccacttcaccaccgcaaaaccaccttacgtgccggaataccgcgcattgctctccctgaaaactgccattacagatgacccacaatctgctcttctttcatggaatatctccacaagtcattgtacatggagaggtgtcacgtgtgaccggtacgtgacttctctcgacatatctggttttaatctcaccggtactcttacgccggaagttggtcatctccgttttttgctcaatctttctgtagctgttaaccagttctctggacccattcctgttgaactctcgtttataccaaatctgcgttaccttaacctctctaacaatattttcaacttgagtttccctccccagcttacccatctccggtacttgaatgttctcgacatttataataacaatatgaccggtgaacttcctgttggattttataatttgaccaatcttcgacatcttcatttgggtggcaatttttttagtggtagtattccaccggagtatggtagattcccattcctagaatatctggcagtttcgggaaatgcgctcgtcggtaggataccaccggagatcggaaatattaccacacttcgtgagctttacatcggatactacaacacgttttccggtgggttaccggcggaaatagggtacttgtcggagctcattcggttagatgctgcaaactgtggactttcaggaggtcacttgcattgggataccaggtataagatagcattggaggctgcaaagggactttgttatctccatcacgattgctcgcctctgatcctccatcgtgatgtaaaatcaaacaatatccttctggattccagcttcgaagcgcacgttgctgattttgggcttgccaagttcttgcaagactccggaacatcagaatgcatgtctgctattgctggttcttatggctacattgcaccagaatatgcatacacactcaaggtagatgagaagagtgatgtatacagctttggtgtggttctgttagaattggtgagcgggaaaaaaccggttggagaatttggtgatggcgttgacatagtccaatgggtaaggaggatgaccgatgggaaaaaggaaggagttctaaagatccttgatgcaagactctcaacagttccccttcatgaggtgatgcatgtgttctatgtcgcaatgctgtgtgtcgaagagcaagctgttgaacgccccaaaatgcgcgaggttgtgcaaatgttaactgagcttcccaagccatctggtccaaaatcaggagattcaacaatcaccgagtcgcccccttcatcaggtcctgcatcagagtctcctacttcgactcccagagacacaaaagaccagtaccatcatcagccaccacctcaatctcctccacctgaccttctcagcatatgacctgaaatgttcacttgtaatagagggtgtagttctcttctttaagttttattagtatcagttttattggggggttggtttattgtttaggctattagcttttcttaggaagtgtctcattgtacagtaagattggcagtaactttatccttcaaatttttccgtttgctttttagctttttgatattgaaagaatcccagtggtcaagctcaccactagccacttttcatcatta